European Patent Application EP 4 467 569 A1, published November 27, 2024. Title: ANTI-B7-H7 ANTIBODY OR ANTIGEN-BINDING FRAGMENT THEREOF, AND PREPARATION METHOD THEREFOR AND USE THEREOF. Applicant: HARBOUR BIOMED(SHANGHAI) CO.,LTD. Application EP 23742894.1, filed January 17, 2023. The sequence listing filed with the application follows.

SEQUENCE LISTING (208 sequences)

SEQ ID NO: 1 - protein, 25 aa, synthetic construct
  REGION 1..25: note = PR003181 HFWR1 Chothia, PR004260 HFWR1 Chothia
QVQLQQSGAELVKPGASVKLSCKAS

SEQ ID NO: 2 - protein, 25 aa, synthetic construct
  REGION 1..25: note = PR003248 HFWR1 Chothia, PR003249 HFWR1 Chothia, PR003250 HFWR1 Chothia
QVQLVESGGGVVQPGRSLRLSCAAS

SEQ ID NO: 3 - protein, 25 aa, synthetic construct
  REGION 1..25: note = PR003251 HFWR1 Chothia
QVQLVESGGGVVQPGRSLRLSCAVS

SEQ ID NO: 4 - protein, 25 aa, synthetic construct
  REGION 1..25: note = PR003260 HFWR1 Chothia
QVQLVESGGGVVQPGRSLRLPCAAS

SEQ ID NO: 5 - protein, 25 aa, synthetic construct
  REGION 1..25: note = PR003264 HFWR1 Chothia, PR004263 HFWR1 Chothia
QVQLVQSGAEVKKPGSSVKVSCKTS

SEQ ID NO: 6 - protein, 7 aa, synthetic construct
  REGION 1..7: note = PR003181 HCDR1 Chothia, PR004260 HCDR1 Chothia
GYTFTSH

SEQ ID NO: 7 - protein, 7 aa, synthetic construct
  REGION 1..7: note = PR003248 HCDR1 Chothia, PR003249 HCDR1 Chothia, PR003250 HCDR1 Chothia
GFTFSDY

SEQ ID NO: 8 - protein, 7 aa, synthetic construct
  REGION 1..7: note = PR003251 HCDR1 Chothia, PR003260 HCDR1 Chothia, PR003262 HCDR1 Chothia
GFTFSRY

SEQ ID NO: 9 - protein, 7 aa, synthetic construct
  REGION 1..7: note = PR003252 HCDR1 Chothia, PR003259 HCDR1 Chothia, PR003261 HCDR1 Chothia
GFTFSNY

SEQ ID NO: 10 - protein, 7 aa, synthetic construct
  REGION 1..7: note = PR003254 HCDR1 Chothia
GFTFSSY

SEQ ID NO: 11 - protein, 7 aa, synthetic construct
  REGION 1..7: note = PR003263 HCDR1 Chothia
GFTFSYY

SEQ ID NO: 12 - protein, 7 aa, synthetic construct
  REGION 1..7: note = PR003264 HCDR1 Chothia, PR004263 HCDR1 Chothia
GGTFSSY

SEQ ID NO: 13 - protein, 7 aa, synthetic construct
  REGION 1..7: note = PR003265 HCDR1 Chothia
GFTFSTY

SEQ ID NO: 14 - protein, 19 aa, synthetic construct
  REGION 1..19: note = PR003181 HFWR2 Chothia, PR004260 HFWR2 Chothia
DINWVRQRPEQGLEWIGWI

SEQ ID NO: 15 - protein, 19 aa, synthetic construct
  REGION 1..19: note = PR003248 HFWR2 Chothia
GLHWVRQAPGRGLEWVAVI

SEQ ID NO: 16 - protein, 19 aa, synthetic construct
  REGION 1..19: note = PR003249 HFWR2 Chothia, PR003250 HFWR2 Chothia, PR003262 HFWR2 Chothia
GIHWVRQAPGKGLEWVAVI

SEQ ID NO: 17 - protein, 19 aa, synthetic construct
  REGION 1..19: note = PR003251 HFWR2 Chothia
GMHWVRQAPGKGLDWVAVI

SEQ ID NO: 18 - protein, 19 aa, synthetic construct
  REGION 1..19: note = PR003252 HFWR2 Chothia
AMHWVRQVPGKGLEWVALI

SEQ ID NO: 19 - protein, 19 aa, synthetic construct
  REGION 1..19: note = PR003254 HFWR2 Chothia, PR003260 HFWR2 Chothia
GMHWVRQAPGKGLEWVADI

SEQ ID NO: 20 - protein, 19 aa, synthetic construct
  REGION 1..19: note = PR003259 HFWR2 Chothia, PR004262 HFWR2 Chothia, PR004487 HFWR2 Chothia
GMHWVRQVPGKGLEWVAVI

SEQ ID NO: 21 - protein, 19 aa, synthetic construct
  REGION 1..19: note = PR003261 HFWR2 Chothia
GMHWVRQAPGKGLEWVAVI

SEQ ID NO: 22 - protein, 19 aa, synthetic construct
  REGION 1..19: note = PR003263 HFWR2 Chothia
GLNWVRQAPGKGLEWVAVI

SEQ ID NO: 23 - protein, 19 aa, synthetic construct
  REGION 1..19: note = PR003264 HFWR2 Chothia, PR004263 HFWR2 Chothia
AISWVRQAPGQGLEWMGGI

SEQ ID NO: 24 - protein, 19 aa, synthetic construct
  REGION 1..19: note = PR003265 HFWR2 Chothia
GLHWVRQAPGKGLEWVAVI

SEQ ID NO: 25 - protein, 19 aa, synthetic construct
  REGION 1..19: note = PR003266 HFWR2 Chothia
GMHWVRQAPGKGLEWVAII

SEQ ID NO: 26 - protein, 6 aa, synthetic construct
  REGION 1..6: note = PR003181 HCDR2 Chothia, PR004260 HCDR2 Chothia
FPGDGS

SEQ ID NO: 27 - protein, 6 aa, synthetic construct
  REGION 1..6: note = PR003248 HCDR2 Chothia, PR003252 HCDR2 Chothia, PR003259 HCDR2 Chothia
WYDGSE

SEQ ID NO: 28 - protein, 6 aa, synthetic construct
  REGION 1..6: note = PR003249 HCDR2 Chothia, PR003250 HCDR2 Chothia, PR004261 HCDR2 Chothia
WYDGSD

SEQ ID NO: 29 - protein, 6 aa, synthetic construct
  REGION 1..6: note = PR003251 HCDR2 Chothia, PR003254 HCDR2 Chothia
WYNGNN

SEQ ID NO: 30 - protein, 6 aa, synthetic construct
  REGION 1..6: note = PR003260 HCDR2 Chothia
WYDGSK

SEQ ID NO: 31 - protein, 6 aa, synthetic construct
  REGION 1..6: note = PR003261 HCDR2 Chothia
WYDGTN

SEQ ID NO: 32 - protein, 6 aa, synthetic construct
  REGION 1..6: note = PR003262 HCDR2 Chothia
WYNGRN

SEQ ID NO: 33 - protein, 6 aa, synthetic construct
  REGION 1..6: note = PR003263 HCDR2 Chothia
WFDGTN

SEQ ID NO: 34 - protein, 6 aa, synthetic construct
  REGION 1..6: note = PR003264 HCDR2 Chothia, PR004263 HCDR2 Chothia
IPLIGT

SEQ ID NO: 35 - protein, 6 aa, synthetic construct
  REGION 1..6: note = PR003265 HCDR2 Chothia
WYDESN

SEQ ID NO: 36 - protein, 6 aa, synthetic construct
  REGION 1..6: note = PR003266 HCDR2 Chothia
WYDGSN

SEQ ID NO: 37 - protein, 6 aa, synthetic construct
  REGION 1..6: note = PR004479 HCDR2 Chothia, PR004480 HCDR2 Chothia, PR004481 HCDR2 Chothia
WYEGSD

SEQ ID NO: 38 - protein, 6 aa, synthetic construct
  REGION 1..6: note = PR004482 HCDR2 Chothia, PR004483 HCDR2 Chothia, PR004484 HCDR2 Chothia
WYDASD

SEQ ID NO: 39 - protein, 6 aa, synthetic construct
  REGION 1..6: note = PR004487 HCDR2 Chothia, PR004488 HCDR2 Chothia, PR004489 HCDR2 Chothia
WYEGSE

SEQ ID NO: 40 - protein, 6 aa, synthetic construct
  REGION 1..6: note = PR004490 HCDR2 Chothia, PR004491 HCDR2 Chothia, PR004492 HCDR2 Chothia
WYDASE

SEQ ID NO: 41 - protein, 41 aa, synthetic construct
  REGION 1..41: note = PR003181 HFWR3 Chothia, PR004260 HFWR3 Chothia
TKFNEKFKGKATLTTDKSSSTAYIQLSRLTSEDSAVYFCAR

SEQ ID NO: 42 - protein, 41 aa, synthetic construct
  REGION 1..41: note = PR003248 HFWR3 Chothia
EYYADSVKGRFTISRDNSKKSLYLQMNSLRAEDTAVYFCAR

SEQ ID NO: 43 - protein, 41 aa, synthetic construct
  REGION 1..41: note = PR003249 HFWR3 Chothia, PR004261 HFWR3 Chothia, PR004479 HFWR3 Chothia
KYYADSVRGRFTISRDNSKNTLSLQMNSLRVEDTAVYYCAR

SEQ ID NO: 44 - protein, 41 aa, synthetic construct
  REGION 1..41: note = PR003250 HFWR3 Chothia
KYYADSVRGRFTISRDNSKNTLSLQMNSLRAEDTAVYYCAR

SEQ ID NO: 45 - protein, 41 aa, synthetic construct
  REGION 1..41: note = PR003251 HFWR3 Chothia
KYYTDSVKGRFTISRDNSKNTLFLQMNSLRAEDTAVYYCAR

SEQ ID NO: 46 - protein, 41 aa, synthetic construct
  REGION 1..41: note = PR003252 HFWR3 Chothia
KYYADSVKGRFTISRDDSKNTLFLQMSSLRAEDTAVYSCVR

SEQ ID NO: 47 - protein, 41 aa, synthetic construct
  REGION 1..41: note = PR003254 HFWR3 Chothia
KYYADSVKGRFTISRDNSKNTLYLQMNSLRAEDTALYYCAR

SEQ ID NO: 48 - protein, 41 aa, synthetic construct
  REGION 1..41: note = PR003259 HFWR3 Chothia, PR004262 HFWR3 Chothia, PR004487 HFWR3 Chothia
KDYADSVKGRFTISRDNSKNTLYLQMNSLRVEDTAVYYCAK

SEQ ID NO: 49 - protein, 41 aa, synthetic construct
  REGION 1..41: note = PR003260 HFWR3 Chothia
KYYADSVKGRFTISRDNSKNTLYLQMNSLRAEDTAVYFCTR

SEQ ID NO: 50 - protein, 41 aa, synthetic construct
  REGION 1..41: note = PR003261 HFWR3 Chothia
KNYADSVKGRFTISRDNSKNTLDLQMNSLRAEDTAVYFCAR

SEQ ID NO: 51 - protein, 41 aa, synthetic construct
  REGION 1..41: note = PR003262 HFWR3 Chothia
KYYVDSVKGRFTISRDNSKNTLYLQMNSLRAEDTAVYYCAR

SEQ ID NO: 52 - protein, 41 aa, synthetic construct
  REGION 1..41: note = PR003263 HFWR3 Chothia
KYYADSVKGRFTISRDDSKNTLYLQMNSLRAEDTAVYYCAR

SEQ ID NO: 53 - protein, 41 aa, synthetic construct
  REGION 1..41: note = PR003264 HFWR3 Chothia, PR004263 HFWR3 Chothia
ANYAQNFQGRVTITADESTRTAYMELSSLRSDDTAVYYCAR

SEQ ID NO: 54 - protein, 41 aa, synthetic construct
  REGION 1..41: note = PR003265 HFWR3 Chothia
EYYADSVKGRFTISRDNSKNTLYLQMNSLRAEDTALYYCAR

SEQ ID NO: 55 - protein, 41 aa, synthetic construct
  REGION 1..41: note = PR003266 HFWR3 Chothia
KYYADSVKGRFTISRDNSKNTLYLQMNSLRAEDTAVYYCAR

SEQ ID NO: 56 - protein, 8 aa, synthetic construct
  REGION 1..8: note = PR003181 HCDR3 Chothia, PR004260 HCDR3 Chothia
NSFYSMDY

SEQ ID NO: 57 - protein, 12 aa, synthetic construct
  REGION 1..12: note = PR003248 HCDR3 Chothia
DRNSGALGYFPH

SEQ ID NO: 58 - protein, 12 aa, synthetic construct
  REGION 1..12: note = PR003249 HCDR3 Chothia, PR004261 HCDR3 Chothia, PR004479 HCDR3 Chothia
DRSSGAMGYFVY

SEQ ID NO: 59 - protein, 12 aa, synthetic construct
  REGION 1..12: note = PR003250 HCDR3 Chothia
DRSSGAMGYFAY

SEQ ID NO: 60 - protein, 11 aa, synthetic construct
  REGION 1..11: note = PR003251 HCDR3 Chothia
DGAYSYGPFDY

SEQ ID NO: 61 - protein, 11 aa, synthetic construct
  REGION 1..11: note = PR003252 HCDR3 Chothia
EYSSGWGYFDY

SEQ ID NO: 62 - protein, 11 aa, synthetic construct
  REGION 1..11: note = PR003254 HCDR3 Chothia, PR003260 HCDR3 Chothia, PR003262 HCDR3 Chothia
DGGYSYGPFDY

SEQ ID NO: 63 - protein, 11 aa, synthetic construct
  REGION 1..11: note = PR003259 HCDR3 Chothia, PR004262 HCDR3 Chothia, PR004487 HCDR3 Chothia
DLISGIYYVDH

SEQ ID NO: 64 - protein, 11 aa, synthetic construct
  REGION 1..11: note = PR003261 HCDR3 Chothia
DRNTAMDYFVY

SEQ ID NO: 65 - protein, 14 aa, synthetic construct
  REGION 1..14: note = PR003263 HCDR3 Chothia
GYGSGSYYNYVMDA

SEQ ID NO: 66 - protein, 12 aa, synthetic construct
  REGION 1..12: note = PR003264 HCDR3 Chothia, PR004263 HCDR3 Chothia
DTMVRGVRALDY

SEQ ID NO: 67 - protein, 12 aa, synthetic construct
  REGION 1..12: note = PR003265 HCDR3 Chothia
LAHDYGGTYFDY

SEQ ID NO: 68 - protein, 12 aa, synthetic construct
  REGION 1..12: note = PR003266 HCDR3 Chothia
DRSSGALGYFQH

SEQ ID NO: 69 - protein, 11 aa, synthetic construct
  REGION 1..11: note = PR003181 HFWR4 Chothia, PR004260 HFWR4 Chothia
WGQGTSVTVSS

SEQ ID NO: 70 - protein, 11 aa, synthetic construct
  REGION 1..11: note = PR003248 HFWR4 Chothia, PR003249 HFWR4 Chothia, PR003250 HFWR4 Chothia
WGQGTLVTVSS

SEQ ID NO: 71 - protein, 11 aa, synthetic construct
  REGION 1..11: note = PR003252 HFWR4 Chothia
WGQGTQVTVSS

SEQ ID NO: 72 - protein, 11 aa, synthetic construct
  REGION 1..11: note = PR003263 HFWR4 Chothia
WGQGASVTVSS

SEQ ID NO: 73 - protein, 23 aa, synthetic construct
  REGION 1..23: note = PR003181 LFWR1 Chothia, PR004260 LFWR1 Chothia
DIVMSQSPSSLAVSAGEKVTMSC

SEQ ID NO: 74 - protein, 23 aa, synthetic construct
  REGION 1..23: note = PR003248 LFWR1 Chothia, PR003249 LFWR1 Chothia, PR003250 LFWR1 Chothia
DIQMTQSPSTLSASVGDRVTITC

SEQ ID NO: 75 - protein, 23 aa, synthetic construct
  REGION 1..23: note = PR003251 LFWR1 Chothia
EIVMTQSPATLSVSPGEGATLSC

SEQ ID NO: 76 - protein, 23 aa, synthetic construct
  REGION 1..23: note = PR003254 LFWR1 Chothia, PR003260 LFWR1 Chothia, PR003262 LFWR1 Chothia
EIVMTQSPATLSVSPGERATLSC

SEQ ID NO: 77 - protein, 23 aa, synthetic construct
  REGION 1..23: note = PR003259 LFWR1 Chothia, PR004262 LFWR1 Chothia, PR004487 LFWR1 Chothia
DIQMTQSPSSLSASVGDRVTITC

SEQ ID NO: 78 - protein, 23 aa, synthetic construct
  REGION 1..23: note = PR003264 LFWR1 Chothia, PR004263 LFWR1 Chothia
DIQLTQSPSFLSASVGDRVTITC

SEQ ID NO: 79 - protein, 23 aa, synthetic construct
  REGION 1..23: note = PR003265 LFWR1 Chothia
EIVMTQSPAILSVSPGERATLSC

SEQ ID NO: 80 - protein, 17 aa, synthetic construct
  REGION 1..17: note = PR003181 LCDR1 Chothia, PR004260 LCDR1 Chothia
KSSQSLLNSRTRKNQLA

SEQ ID NO: 81 - protein, 11 aa, synthetic construct
  REGION 1..11: note = PR003248 LCDR1 Chothia
RASQSINNWLA

SEQ ID NO: 82 - protein, 11 aa, synthetic construct
  REGION 1..11: note = PR003249 LCDR1 Chothia, PR003250 LCDR1 Chothia, PR003252 LCDR1 Chothia
RASQSISSWLA

SEQ ID NO: 83 - protein, 11 aa, synthetic construct
  REGION 1..11: note = PR003251 LCDR1 Chothia, PR003260 LCDR1 Chothia, PR003263 LCDR1 Chothia
RASQSVSSNLA

SEQ ID NO: 84 - protein, 11 aa, synthetic construct
  REGION 1..11: note = PR003254 LCDR1 Chothia
RASQSVSSYLA

SEQ ID NO: 85 - protein, 11 aa, synthetic construct
  REGION 1..11: note = PR003259 LCDR1 Chothia, PR004262 LCDR1 Chothia, PR004487 LCDR1 Chothia
RASQGISNYLA

SEQ ID NO: 86 - protein, 11 aa, synthetic construct
  REGION 1..11: note = PR003262 LCDR1 Chothia
RASQSFSNNLA

SEQ ID NO: 87 - protein, 11 aa, synthetic construct
  REGION 1..11: note = PR003264 LCDR1 Chothia, PR004263 LCDR1 Chothia
RASQGISSYFA

SEQ ID NO: 88 - protein, 11 aa, synthetic construct
  REGION 1..11: note = PR003265 LCDR1 Chothia
RASQSISYNLA

SEQ ID NO: 89 - protein, 15 aa, synthetic construct
  REGION 1..15: note = PR003181 LFWR2 Chothia, PR004260 LFWR2 Chothia
WYQQKPGQSPKLLIY

SEQ ID NO: 90 - protein, 15 aa, synthetic construct
  REGION 1..15: note = PR003248 LFWR2 Chothia, PR003249 LFWR2 Chothia, PR003250 LFWR2 Chothia
WYQQKPGKAPKLLIY

SEQ ID NO: 91 - protein, 15 aa, synthetic construct
  REGION 1..15: note = PR003251 LFWR2 Chothia, PR003254 LFWR2 Chothia, PR003260 LFWR2 Chothia
WYQQKPGQAPRLLIY

SEQ ID NO: 92 - protein, 15 aa, synthetic construct
  REGION 1..15: note = PR003259 LFWR2 Chothia, PR004262 LFWR2 Chothia, PR004487 LFWR2 Chothia
WYQQKPGKVPKLLIY

SEQ ID NO: 93 - protein, 7 aa, synthetic construct
  REGION 1..7: note = PR003181 LCDR2 Chothia, PR004260 LCDR2 Chothia
WASTRES

SEQ ID NO: 94 - protein, 7 aa, synthetic construct
  REGION 1..7: note = PR003248 LCDR2 Chothia, PR003249 LCDR2 Chothia, PR003250 LCDR2 Chothia
KASSLES

SEQ ID NO: 95 - protein, 7 aa, synthetic construct
  REGION 1..7: note = PR003251 LCDR2 Chothia, PR003254 LCDR2 Chothia, PR003262 LCDR2 Chothia
GASTRAT

SEQ ID NO: 96 - protein, 7 aa, synthetic construct
  REGION 1..7: note = PR003252 LCDR2 Chothia
KASSLKS

SEQ ID NO: 97 - protein, 7 aa, synthetic construct
  REGION 1..7: note = PR003259 LCDR2 Chothia, PR003264 LCDR2 Chothia, PR004262 LCDR2 Chothia
AASTLQS

SEQ ID NO: 98 - protein, 7 aa, synthetic construct
  REGION 1..7: note = PR003260 LCDR2 Chothia
YASTRAP

SEQ ID NO: 99 - protein, 7 aa, synthetic construct
  REGION 1..7: note = PR003263 LCDR2 Chothia
GASTGAT

SEQ ID NO: 100 - protein, 7 aa, synthetic construct
  REGION 1..7: note = PR003265 LCDR2 Chothia
GASIRAT

SEQ ID NO: 101 - protein, 32 aa, synthetic construct
  REGION 1..32: note = PR003181 LFWR3 Chothia, PR004260 LFWR3 Chothia
GVPDRFTGSGSGTDFTLTISSVQAEDLAVYYC

SEQ ID NO: 102 - protein, 32 aa, synthetic construct
  REGION 1..32: note = PR003248 LFWR3 Chothia, PR003252 LFWR3 Chothia, PR003266 LFWR3 Chothia
GVPSRFSGSGSGTEFTLTISSLQPDDFATYYC

SEQ ID NO: 103 - protein, 32 aa, synthetic construct
  REGION 1..32: note = PR003249 LFWR3 Chothia, PR003250 LFWR3 Chothia, PR004261 LFWR3 Chothia
GVPSRFSGSGSGTEFTLTISSLQPDDLATYYC

SEQ ID NO: 104 - protein, 32 aa, synthetic construct
  REGION 1..32: note = PR003251 LFWR3 Chothia, PR003254 LFWR3 Chothia, PR003262 LFWR3 Chothia
GIPARFSGSGSGTEFTLTISSLQSEDFAVYYC

SEQ ID NO: 105 - protein, 32 aa, synthetic construct
  REGION 1..32: note = PR003259 LFWR3 Chothia, PR004262 LFWR3 Chothia, PR004487 LFWR3 Chothia
GVPSRFSGSGSGTDFTLTISSLQPEDVATYYC

SEQ ID NO: 106 - protein, 32 aa, synthetic construct
  REGION 1..32: note = PR003260 LFWR3 Chothia
GIPARFSGSESGTEFTLTISSLQSEDFAVYYC

SEQ ID NO: 107 - protein, 32 aa, synthetic construct
  REGION 1..32: note = PR003261 LFWR3 Chothia
GVPSRFSGSGSGTEFTLTISSLQPDDFASYYC

SEQ ID NO: 108 - protein, 32 aa, synthetic construct
  REGION 1..32: note = PR003263 LFWR3 Chothia, PR003265 LFWR3 Chothia
GIPARFSGSGSGTDFTLTISSLQSEDFAVYYC

SEQ ID NO: 109 - protein, 32 aa, synthetic construct
  REGION 1..32: note = PR003264 LFWR3 Chothia, PR004263 LFWR3 Chothia
GVPSRFSGSGSGTEFTLTISSLQPEDFATYYC

SEQ ID NO: 110 - protein, 8 aa, synthetic construct
  REGION 1..8: note = PR003181 LCDR3 Chothia, PR004260 LCDR3 Chothia
KQSYNLRT

SEQ ID NO: 111 - protein, 8 aa, synthetic construct
  REGION 1..8: note = PR003248 LCDR3 Chothia, PR003266 LCDR3 Chothia
QQYNSYST

SEQ ID NO: 112 - protein, 9 aa, synthetic construct
  REGION 1..9: note = PR003249 LCDR3 Chothia, PR003250 LCDR3 Chothia, PR004261 LCDR3 Chothia
QQYNSYSYT

SEQ ID NO: 113 - protein, 9 aa, synthetic construct
  REGION 1..9: note = PR003251 LCDR3 Chothia, PR003260 LCDR3 Chothia
QQYNIWPYT

SEQ ID NO: 114 - protein, 8 aa, synthetic construct
  REGION 1..8: note = PR003252 LCDR3 Chothia
LQYNSYYT

SEQ ID NO: 115 - protein, 9 aa, synthetic construct
  REGION 1..9: note = PR003254 LCDR3 Chothia
QQYNNWPLT

SEQ ID NO: 116 - protein, 9 aa, synthetic construct
  REGION 1..9: note = PR003259 LCDR3 Chothia, PR004262 LCDR3 Chothia, PR004487 LCDR3 Chothia
QKYNSAPFT

SEQ ID NO: 117 - protein, 9 aa, synthetic construct
  REGION 1..9: note = PR003261 LCDR3 Chothia
QQYNSYSVT

SEQ ID NO: 118 - protein, 9 aa, synthetic construct
  REGION 1..9: note = PR003262 LCDR3 Chothia
HQYNIWPLT

SEQ ID NO: 119 - protein, 9 aa, synthetic construct
  REGION 1..9: note = PR003263 LCDR3 Chothia
QQYYKWPLT

SEQ ID NO: 120 - protein, 9 aa, synthetic construct
  REGION 1..9: note = PR003264 LCDR3 Chothia, PR004263 LCDR3 Chothia
QHLNRYPWT

SEQ ID NO: 121 - protein, 10 aa, synthetic construct [sequence omitted]

SEQ ID NO: 122 - protein, 9 aa, synthetic construct
  REGION 1..9: note = PR004480 LCDR3 Chothia, PR004483 LCDR3 Chothia, PR004485 LCDR3 Chothia
QQYQSYSYT

SEQ ID NO: 123 - protein, 9 aa, synthetic construct
  REGION 1..9: note = PR004481 LCDR3 Chothia, PR004484 LCDR3 Chothia, PR004486 LCDR3 Chothia
QQYNAYSYT

SEQ ID NO: 124 - protein, 9 aa, synthetic construct
  REGION 1..9: note = PR004488 LCDR3 Chothia, PR004491 LCDR3 Chothia, PR004493 LCDR3 Chothia
QKYQSAPFT

SEQ ID NO: 125 - protein, 9 aa, synthetic construct
  REGION 1..9: note = PR004489 LCDR3 Chothia, PR004492 LCDR3 Chothia, PR004494 LCDR3 Chothia
QKYNAAPFT

SEQ ID NO: 126 - protein, 10 aa, synthetic construct
  REGION 1..10: note = PR003181 LFWR4 Chothia, PR004260 LFWR4 Chothia
FGGGTKLEIK

SEQ ID NO: 127 - protein, 10 aa, synthetic construct
  REGION 1..10: note = PR003248 LFWR4 Chothia, PR003249 LFWR4 Chothia, PR003250 LFWR4 Chothia
FGQGTKLEIK

SEQ ID NO: 128 - protein, 10 aa, synthetic construct
  REGION 1..10: note = PR003254 LFWR4 Chothia, PR003261 LFWR4 Chothia, PR003262 LFWR4 Chothia
FGGGTKVEIK

SEQ ID NO: 129 - protein, 10 aa, synthetic construct
  REGION 1..10: note = PR003259 LFWR4 Chothia, PR004262 LFWR4 Chothia, PR004487 LFWR4 Chothia
FGPGTKVDIK

SEQ ID NO: 130 - protein, 10 aa, synthetic construct
  REGION 1..10: note = PR003264 LFWR4 Chothia, PR003265 LFWR4 Chothia, PR004263 LFWR4 Chothia
FGQGTKVEIK

SEQ ID NO: 131 - protein, 117 aa, synthetic construct
  REGION 1..117: note = PR003181 VH, PR004260 VH
QVQLQQSGAELVKPGASVKLSCKASGYTFTSHDINWVRQRPEQGLEWIGWIFPGDGSTKFNEKFKGKATLTTDKSSSTAYIQLSRLTSEDSAVYFCARNSFYSMDYWGQGTSVTVSS

SEQ ID NO: 132 - protein, 121 aa, synthetic construct
  REGION 1..121: note = PR003248 VH
QVQLVESGGGVVQPGRSLRLSCAASGFTFSDYGLHWVRQAPGRGLEWVAVIWYDGSEEYYADSVKGRFTISRDNSKKSLYLQMNSLRAEDTAVYFCARDRNSGALGYFPHWGQGTLVTVSS

SEQ ID NO: 133 - protein, 121 aa, synthetic construct
  REGION 1..121: note = PR003249 VH, PR004261 VH, PR004485 VH, PR004486 VH
QVQLVESGGGVVQPGRSLRLSCAASGFTFSDYGIHWVRQAPGKGLEWVAVIWYDGSDKYYADSVRGRFTISRDNSKNTLSLQMNSLRVEDTAVYYCARDRSSGAMGYFVYWGQGTLVTVSS

SEQ ID NO: 134 - protein, 121 aa, synthetic construct
  REGION 1..121: note = PR003250 VH
QVQLVESGGGVVQPGRSLRLSCAASGFTFSDYGIHWVRQAPGKGLEWVAVIWYDGSDKYYADSVRGRFTISRDNSKNTLSLQMNSLRAEDTAVYYCARDRSSGAMGYFAYWGQGTLVTVSS

SEQ ID NO: 135 - protein, 120 aa, synthetic construct
  REGION 1..120: note = PR003251 VH
QVQLVESGGGVVQPGRSLRLSCAVSGFTFSRYGMHWVRQAPGKGLDWVAVIWYNGNNKYYTDSVKGRFTISRDNSKNTLFLQMNSLRAEDTAVYYCARDGAYSYGPFDYWGQGTLVTVSS

SEQ ID NO: 136 - protein, 120 aa, synthetic construct
  REGION 1..120: note = PR003252 VH
QVQLVESGGGVVQPGRSLRLSCAASGFTFSNYAMHWVRQVPGKGLEWVALIWYDGSEKYYADSVKGRFTISRDDSKNTLFLQMSSLRAEDTAVYSCVREYSSGWGYFDYWGQGTQVTVSS

SEQ ID NO: 137 - protein, 120 aa, synthetic construct
  REGION 1..120: note = PR003254 VH
QVQLVESGGGVVQPGRSLRLSCAASGFTFSSYGMHWVRQAPGKGLEWVADIWYNGNNKYYADSVKGRFTISRDNSKNTLYLQMNSLRAEDTALYYCARDGGYSYGPFDYWGQGTLVTVSS

SEQ ID NO: 138 - protein, 120 aa, synthetic construct
  REGION 1..120: note = PR003259 VH, PR004262 VH, PR004493 VH, PR004494 VH
QVQLVESGGGVVQPGRSLRLSCAASGFTFSNYGMHWVRQVPGKGLEWVAVIWYDGSEKDYADSVKGRFTISRDNSKNTLYLQMNSLRVEDTAVYYCAKDLISGIYYVDHWGQGTLVTVSS

SEQ ID NO: 139 - protein, 120 aa, synthetic construct
  REGION 1..120: note = PR003260 VH
QVQLVESGGGVVQPGRSLRLPCAASGFTFSRYGMHWVRQAPGKGLEWVADIWYDGSKKYYADSVKGRFTISRDNSKNTLYLQMNSLRAEDTAVYFCTRDGGYSYGPFDYWGQGTLVTVSS

SEQ ID NO: 140 - protein, 120 aa, synthetic construct
  REGION 1..120: note = PR003261 VH
QVQLVESGGGVVQPGRSLRLSCAASGFTFSNYGMHWVRQAPGKGLEWVAVIWYDGTNKNYADSVKGRFTISRDNSKNTLDLQMNSLRAEDTAVYFCARDRNTAMDYFVYWGQGTLVTVSS

SEQ ID NO: 141 - protein, 120 aa, synthetic construct
  REGION 1..120: note = PR003262 VH
QVQLVESGGGVVQPGRSLRLSCAASGFTFSRYGIHWVRQAPGKGLEWVAVIWYNGRNKYYVDSVKGRFTISRDNSKNTLYLQMNSLRAEDTAVYYCARDGGYSYGPFDYWGQGTLVTVSS

SEQ ID NO: 142 - protein, 123 aa, synthetic construct
  REGION 1..123: note = PR003263 VH
QVQLVESGGGVVQPGRSLRLSCAASGFTFSYYGLNWVRQAPGKGLEWVAVIWFDGTNKYYADSVKGRFTISRDDSKNTLYLQMNSLRAEDTAVYYCARGYGSGSYYNYVMDAWGQGASVTVSS

SEQ ID NO: 143 - protein, 121 aa, synthetic construct
  REGION 1..121: note = PR003264 VH, PR004263 VH
QVQLVQSGAEVKKPGSSVKVSCKTSGGTFSSYAISWVRQAPGQGLEWMGGIIPLIGTANYAQNFQGRVTITADESTRTAYMELSSLRSDDTAVYYCARDTMVRGVRALDYWGQGTLVTVSS

SEQ ID NO: 144 - protein, 121 aa, synthetic construct
  REGION 1..121: note = PR003265 VH
QVQLVESGGGVVQPGRSLRLSCAASGFTFSTYGLHWVRQAPGKGLEWVAVIWYDESNEYYADSVKGRFTISRDNSKNTLYLQMNSLRAEDTALYYCARLAHDYGGTYFDYWGQGTLVTVSS

SEQ ID NO: 145 - protein, 121 aa, synthetic construct
  REGION 1..121: note = PR003266 VH
QVQLVESGGGVVQPGRSLRLSCAASGFTFSDYGMHWVRQAPGKGLEWVAIIWYDGSNKYYADSVKGRFTISRDNSKNTLYLQMNSLRAEDTAVYYCARDRSSGALGYFQHWGQGTLVTVSS

SEQ ID NO: 146 - protein, 121 aa, synthetic construct
  REGION 1..121: note = PR004479 VH, PR004480 VH, PR004481 VH
QVQLVESGGGVVQPGRSLRLSCAASGFTFSDYGIHWVRQAPGKGLEWVAVIWYEGSDKYYADSVRGRFTISRDNSKNTLSLQMNSLRVEDTAVYYCARDRSSGAMGYFVYWGQGTLVTVSS

SEQ ID NO: 147 - protein, 121 aa, synthetic construct
  REGION 1..121: note = PR004482 VH, PR004483 VH, PR004484 VH
QVQLVESGGGVVQPGRSLRLSCAASGFTFSDYGIHWVRQAPGKGLEWVAVIWYDASDKYYADSVRGRFTISRDNSKNTLSLQMNSLRVEDTAVYYCARDRSSGAMGYFVYWGQGTLVTVSS

SEQ ID NO: 148 - protein, 120 aa, synthetic construct
  REGION 1..120: note = PR004487 VH, PR004488 VH, PR004489 VH
QVQLVESGGGVVQPGRSLRLSCAASGFTFSNYGMHWVRQVPGKGLEWVAVIWYEGSEKDYADSVKGRFTISRDNSKNTLYLQMNSLRVEDTAVYYCAKDLISGIYYVDHWGQGTLVTVSS

SEQ ID NO: 149 - protein, 120 aa, synthetic construct
  REGION 1..120: note = PR004490 VH, PR004491 VH, PR004492 VH
QVQLVESGGGVVQPGRSLRLSCAASGFTFSNYGMHWVRQVPGKGLEWVAVIWYDASEKDYADSVKGRFTISRDNSKNTLYLQMNSLRVEDTAVYYCAKDLISGIYYVDHWGQGTLVTVSS

SEQ ID NO: 150 - protein, 112 aa, synthetic construct
  REGION 1..112: note = PR003181 VL, PR004260 VL
DIVMSQSPSSLAVSAGEKVTMSCKSSQSLLNSRTRKNQLAWYQQKPGQSPKLLIYWASTRESGVPDRFTGSGSGTDFTLTISSVQAEDLAVYYCKQSYNLRTFGGGTKLEIK

SEQ ID NO: 151 - protein, 106 aa, synthetic construct
  REGION 1..106: note = PR003248 VL
DIQMTQSPSTLSASVGDRVTITCRASQSINNWLAWYQQKPGKAPKLLIYKASSLESGVPSRFSGSGSGTEFTLTISSLQPDDFATYYCQQYNSYSTFGQGTKLEIK

SEQ ID NO: 152 - protein, 107 aa, synthetic construct
  REGION 1..107: note = PR003249 VL, PR003250 VL, PR004261 VL, PR004479 VL, PR004482 VL
DIQMTQSPSTLSASVGDRVTITCRASQSISSWLAWYQQKPGKAPKLLIYKASSLESGVPSRFSGSGSGTEFTLTISSLQPDDLATYYCQQYNSYSYTFGQGTKLEIK

SEQ ID NO: 153 - protein, 107 aa, synthetic construct
  REGION 1..107: note = PR003251 VL
EIVMTQSPATLSVSPGEGATLSCRASQSVSSNLAWYQQKPGQAPRLLIYGASTRATGIPARFSGSGSGTEFTLTISSLQSEDFAVYYCQQYNIWPYTFGQGTKLEIK

SEQ ID NO: 154 - protein, 106 aa, synthetic construct
  REGION 1..106: note = PR003252 VL
DIQMTQSPSTLSASVGDRVTITCRASQSISSWLAWYQQKPGKAPKLLIYKASSLKSGVPSRFSGSGSGTEFTLTISSLQPDDFATYYCLQYNSYYTFGQGTKLEIK

SEQ ID NO: 155 - protein, 107 aa, synthetic construct
  REGION 1..107: note = PR003254 VL
EIVMTQSPATLSVSPGERATLSCRASQSVSSYLAWYQQKPGQAPRLLIYGASTRATGIPARFSGSGSGTEFTLTISSLQSEDFAVYYCQQYNNWPLTFGGGTKVEIK

SEQ ID NO: 156 - protein, 107 aa, synthetic construct
  REGION 1..107: note = PR003259 VL, PR004262 VL, PR004487 VL, PR004490 VL
DIQMTQSPSSLSASVGDRVTITCRASQGISNYLAWYQQKPGKVPKLLIYAASTLQSGVPSRFSGSGSGTDFTLTISSLQPEDVATYYCQKYNSAPFTFGPGTKVDIK

SEQ ID NO: 157 - protein, 107 aa, synthetic construct
  REGION 1..107: note = PR003260 VL
EIVMTQSPATLSVSPGERATLSCRASQSVSSNLAWYQQKPGQAPRLLIYYASTRAPGIPARFSGSESGTEFTLTISSLQSEDFAVYYCQQYNIWPYTFGQGTKLEIK

SEQ ID NO: 158 - protein, 107 aa, synthetic construct
  REGION 1..107: note = PR003261 VL
DIQMTQSPSTLSASVGDRVTITCRASQSISSWLAWYQQKPGKAPKLLIYKASSLESGVPSRFSGSGSGTEFTLTISSLQPDDFASYYCQQYNSYSVTFGGGTKVEIK

SEQ ID NO: 159 - protein, 107 aa, synthetic construct
  REGION 1..107: note = PR003262 VL
EIVMTQSPATLSVSPGERATLSCRASQSFSNNLAWYQQKPGQAPRLLIYGASTRATGIPARFSGSGSGTEFTLTISSLQSEDFAVYYCHQYNIWPLTFGGGTKVEIK

SEQ ID NO: 160 - protein, 107 aa, synthetic construct
  REGION 1..107: note = PR003263 VL
EIVMTQSPATLSVSPGERATLSCRASQSVSSNLAWYQQKPGQAPRLLIYGASTGATGIPARFSGSGSGTDFTLTISSLQSEDFAVYYCQQYYKWPLTFGGGTKVEIK

SEQ ID NO: 161 - protein, 107 aa, synthetic construct
  REGION 1..107: note = PR003264 VL, PR004263 VL
DIQLTQSPSFLSASVGDRVTITCRASQGISSYFAWYQQKPGKAPKLLIYAASTLQSGVPSRFSGSGSGTEFTLTISSLQPEDFATYYCQHLNRYPWTFGQGTKVEIK

SEQ ID NO: 162 - protein, 108 aa, synthetic construct
  REGION 1..108: note = PR003265 VL
EIVMTQSPAILSVSPGERATLSCRASQSISYNLAWYQQKPGQAPRLLIYGASIRATGIPARFSGSGSGTDFTLTISSLQSEDFAVYYCQQYNNWPPWTFGQGTKVEIK

SEQ ID NO: 163 - protein, 106 aa, synthetic construct
  REGION 1..106: note = PR003266 VL
DIQMTQSPSTLSASVGDRVTITCRASQSISSWLAWYQQKPGKAPKLLIYKASSLESGVPSRFSGSGSGTEFTLTISSLQPDDFATYYCQQYNSYSTFGQGTKLEIK

SEQ ID NO: 164 - protein, 107 aa, synthetic construct
  REGION 1..107: note = PR004480 VL, PR004483 VL, PR004485 VL
DIQMTQSPSTLSASVGDRVTITCRASQSISSWLAWYQQKPGKAPKLLIYKASSLESGVPSRFSGSGSGTEFTLTISSLQPDDLATYYCQQYQSYSYTFGQGTKLEIK

SEQ ID NO: 165 - protein, 107 aa, synthetic construct
  REGION 1..107: note = PR004481 VL, PR004484 VL, PR004486 VL
DIQMTQSPSTLSASVGDRVTITCRASQSISSWLAWYQQKPGKAPKLLIYKASSLESGVPSRFSGSGSGTEFTLTISSLQPDDLATYYCQQYNAYSYTFGQGTKLEIK

SEQ ID NO: 166 - protein, 107 aa, synthetic construct
  REGION 1..107: note = PR004488 VL, PR004491 VL, PR004493 VL
DIQMTQSPSSLSASVGDRVTITCRASQGISNYLAWYQQKPGKVPKLLIYAASTLQSGVPSRFSGSGSGTDFTLTISSLQPEDVATYYCQKYQSAPFTFGPGTKVDIK

SEQ ID NO: 167 - protein, 107 aa, synthetic construct
  REGION 1..107: note = PR004489 VL, PR004492 VL, PR004494 VL
DIQMTQSPSSLSASVGDRVTITCRASQGISNYLAWYQQKPGKVPKLLIYAASTLQSGVPSRFSGSGSGTDFTLTISSLQPEDVATYYCQKYNAAPFTFGPGTKVDIK

SEQ ID NO: 168 - protein, 444 aa, synthetic construct
  REGION 1..444: note = PR003181 HC
QVQLQQSGAELVKPGASVKLSCKASGYTFTSHDINWVRQRPEQGLEWIGWIFPGDGSTKFNEKFKGKATLTTDKSSSTAYIQLSRLTSEDSAVYFCARNSFYSMDYWGQGTSVTVSSASTKGPSVFPLAPCSRSTSESTAALGCLVKDYFPEPVTVSWNSGALTSGVHTFPAVLQSSGLYSLSSVVTVPSSSLGTKTYTCNVDHKPSNTKVDKRVESKYGPPCPPCPAPEFLGGPSVFLFPPKPKDTLMISRTPEVTCVVVDVSQEDPEVQFNWYVDGVEVHNAKTKPREEQFNSTYRVVSVLTVLHQDWLNGKEYKCKVSNKGLPSSIEKTISKAKGQPREPQVYTLPPSQEEMTKNQVSLTCLVKGFYPSDIAVEWESNGQPENNYKTTPPVLDSDGSFFLYSRLTVDKSRWQEGNVFSCSVMHEALHNHYTQKSLSLSLGK

SEQ ID NO: 169 - protein, 451 aa, synthetic construct
  REGION 1..451: note = PR003248 HC
QVQLVESGGGVVQPGRSLRLSCAASGFTFSDYGLHWVRQAPGRGLEWVAVIWYDGSEEYYADSVKGRFTISRDNSKKSLYLQMNSLRAEDTAVYFCARDRNSGALGYFPHWGQGTLVTVSSASTKGPSVFPLAPSSKSTSGGTAALGCLVKDYFPEPVTVSWNSGALTSGVHTFPAVLQSSGLYSLSSVVTVPSSSLGTQTYICNVNHKPSNTKVDKKVEPKSCDKTHTCPPCPAPELLGGPSVFLFPPKPKDTLMISRTPEVTCVVVDVSHEDPEVKFNWYVDGVEVHNAKTKPREEQYNSTYRVVSVLTVLHQDWLNGKEYKCKVSNKALPAPIEKTISKAKGQPREPQVYTLPPSREEMTKNQVSLTCLVKGFYPSDIAVEWESNGQPENNYKTTPPVLDSDGSFFLYSKLTVDKSRWQQGNVFSCSVMHEALHNHYTQKSLSLSPGK

SEQ ID NO: 170 - protein, 451 aa, synthetic construct
  REGION 1..451: note = PR003249 HC
QVQLVESGGGVVQPGRSLRLSCAASGFTFSDYGIHWVRQAPGKGLEWVAVIWYDGSDKYYADSVRGRFTISRDNSKNTLSLQMNSLRVEDTAVYYCARDRSSGAMGYFVYWGQGTLVTVSSASTKGPSVFPLAPSSKSTSGGTAALGCLVKDYFPEPVTVSWNSGALTSGVHTFPAVLQSSGLYSLSSVVTVPSSSLGTQTYICNVNHKPSNTKVDKKVEPKSCDKTHTCPPCPAPELLGGPSVFLFPPKPKDTLMISRTPEVTCVVVDVSHEDPEVKFNWYVDGVEVHNAKTKPREEQYNSTYRVVSVLTVLHQDWLNGKEYKCKVSNKALPAPIEKTISKAKGQPREPQVYTLPPSREEMTKNQVSLTCLVKGFYPSDIAVEWESNGQPENNYKTTPPVLDSDGSFFLYSKLTVDKSRWQQGNVFSCSVMHEALHNHYTQKSLSLSPGK

SEQ ID NO: 171 - protein, 451 aa, synthetic construct
  REGION 1..451: note = PR003250 HC
QVQLVESGGGVVQPGRSLRLSCAASGFTFSDYGIHWVRQAPGKGLEWVAVIWYDGSDKYYADSVRGRFTISRDNSKNTLSLQMNSLRAEDTAVYYCARDRSSGAMGYFAYWGQGTLVTVSSASTKGPSVFPLAPSSKSTSGGTAALGCLVKDYFPEPVTVSWNSGALTSGVHTFPAVLQSSGLYSLSSVVTVPSSSLGTQTYICNVNHKPSNTKVDKKVEPKSCDKTHTCPPCPAPELLGGPSVFLFPPKPKDTLMISRTPEVTCVVVDVSHEDPEVKFNWYVDGVEVHNAKTKPREEQYNSTYRVVSVLTVLHQDWLNGKEYKCKVSNKALPAPIEKTISKAKGQPREPQVYTLPPSREEMTKNQVSLTCLVKGFYPSDIAVEWESNGQPENNYKTTPPVLDSDGSFFLYSKLTVDKSRWQQGNVFSCSVMHEALHNHYTQKSLSLSPGK

SEQ ID NO: 172 - protein, 450 aa, synthetic construct
  REGION 1..450: note = PR003251 HC
QVQLVESGGGVVQPGRSLRLSCAVSGFTFSRYGMHWVRQAPGKGLDWVAVIWYNGNNKYYTDSVKGRFTISRDNSKNTLFLQMNSLRAEDTAVYYCARDGAYSYGPFDYWGQGTLVTVSSASTKGPSVFPLAPSSKSTSGGTAALGCLVKDYFPEPVTVSWNSGALTSGVHTFPAVLQSSGLYSLSSVVTVPSSSLGTQTYICNVNHKPSNTKVDKKVEPKSCDKTHTCPPCPAPELLGGPSVFLFPPKPKDTLMISRTPEVTCVVVDVSHEDPEVKFNWYVDGVEVHNAKTKPREEQYNSTYRVVSVLTVLHQDWLNGKEYKCKVSNKALPAPIEKTISKAKGQPREPQVYTLPPSREEMTKNQVSLTCLVKGFYPSDIAVEWESNGQPENNYKTTPPVLDSDGSFFLYSKLTVDKSRWQQGNVFSCSVMHEALHNHYTQKSLSLSPGK

SEQ ID NO: 173 - protein, 450 aa, synthetic construct
  REGION 1..450: note = PR003252 HC
QVQLVESGGGVVQPGRSLRLSCAASGFTFSNYAMHWVRQVPGKGLEWVALIWYDGSEKYYADSVKGRFTISRDDSKNTLFLQMSSLRAEDTAVYSCVREYSSGWGYFDYWGQGTQVTVSSASTKGPSVFPLAPSSKSTSGGTAALGCLVKDYFPEPVTVSWNSGALTSGVHTFPAVLQSSGLYSLSSVVTVPSSSLGTQTYICNVNHKPSNTKVDKKVEPKSCDKTHTCPPCPAPELLGGPSVFLFPPKPKDTLMISRTPEVTCVVVDVSHEDPEVKFNWYVDGVEVHNAKTKPREEQYNSTYRVVSVLTVLHQDWLNGKEYKCKVSNKALPAPIEKTISKAKGQPREPQVYTLPPSREEMTKNQVSLTCLVKGFYPSDIAVEWESNGQPENNYKTTPPVLDSDGSFFLYSKLTVDKSRWQQGNVFSCSVMHEALHNHYTQKSLSLSPGK

SEQ ID NO: 174 - protein, 450 aa, synthetic construct
  REGION 1..450: note = PR003254 HC
QVQLVESGGGVVQPGRSLRLSCAASGFTFSSYGMHWVRQAPGKGLEWVADIWYNGNNKYYADSVKGRFTISRDNSKNTLYLQMNSLRAEDTALYYCARDGGYSYGPFDYWGQGTLVTVSSASTKGPSVFPLAPSSKSTSGGTAALGCLVKDYFPEPVTVSWNSGALTSGVHTFPAVLQSSGLYSLSSVVTVPSSSLGTQTYICNVNHKPSNTKVDKKVEPKSCDKTHTCPPCPAPELLGGPSVFLFPPKPKDTLMISRTPEVTCVVVDVSHEDPEVKFNWYVDGVEVHNAKTKPREEQYNSTYRVVSVLTVLHQDWLNGKEYKCKVSNKALPAPIEKTISKAKGQPREPQVYTLPPSREEMTKNQVSLTCLVKGFYPSDIAVEWESNGQPENNYKTTPPVLDSDGSFFLYSKLTVDKSRWQQGNVFSCSVMHEALHNHYTQKSLSLSPGK

SEQ ID NO: 175 - protein, 450 aa, synthetic construct
  REGION 1..450: note = PR003259 HC
QVQLVESGGGVVQPGRSLRLSCAASGFTFSNYGMHWVRQVPGKGLEWVAVIWYDGSEKDYADSVKGRFTISRDNSKNTLYLQMNSLRVEDTAVYYCAKDLISGIYYVDHWGQGTLVTVSSASTKGPSVFPLAPSSKSTSGGTAALGCLVKDYFPEPVTVSWNSGALTSGVHTFPAVLQSSGLYSLSSVVTVPSSSLGTQTYICNVNHKPSNTKVDKKVEPKSCDKTHTCPPCPAPELLGGPSVFLFPPKPKDTLMISRTPEVTCVVVDVSHEDPEVKFNWYVDGVEVHNAKTKPREEQYNSTYRVVSVLTVLHQDWLNGKEYKCKVSNKALPAPIEKTISKAKGQPREPQVYTLPPSREEMTKNQVSLTCLVKGFYPSDIAVEWESNGQPENNYKTTPPVLDSDGSFFLYSKLTVDKSRWQQGNVFSCSVMHEALHNHYTQKSLSLSPGK

SEQ ID NO: 176 - protein, 450 aa, synthetic construct
  REGION 1..450: note = PR003260 HC
QVQLVESGGGVVQPGRSLRLPCAASGFTFSRYGMHWVRQAPGKGLEWVADIWYDGSKKYYADSVKGRFTISRDNSKNTLYLQMNSLRAEDTAVYFCTRDGGYSYGPFDYWGQGTLVTVSSASTKGPSVFPLAPSSKSTSGGTAALGCLVKDYFPEPVTVSWNSGALTSGVHTFPAVLQSSGLYSLSSVVTVPSSSLGTQTYICNVNHKPSNTKVDKKVEPKSCDKTHTCPPCPAPELLGGPSVFLFPPKPKDTLMISRTPEVTCVVVDVSHEDPEVKFNWYVDGVEVHNAKTKPREEQYNSTYRVVSVLTVLHQDWLNGKEYKCKVSNKALPAPIEKTISKAKGQPREPQVYTLPPSREEMTKNQVSLTCLVKGFYPSDIAVEWESNGQPENNYKTTPPVLDSDGSFFLYSKLTVDKSRWQQGNVFSCSVMHEALHNHYTQKSLSLSPGK

SEQ ID NO: 177 - protein, 450 aa, synthetic construct
  REGION 1..450: note = PR003261 HC
QVQLVESGGGVVQPGRSLRLSCAASGFTFSNYGMHWVRQAPGKGLEWVAVIWYDGTNKNYADSVKGRFTISRDNSKNTLDLQMNSLRAEDTAVYFCARDRNTAMDYFVYWGQGTLVTVSSASTKGPSVFPLAPSSKSTSGGTAALGCLVKDYFPEPVTVSWNSGALTSGVHTFPAVLQSSGLYSLSSVVTVPSSSLGTQTYICNVNHKPSNTKVDKKVEPKSCDKTHTCPPCPAPELLGGPSVFLFPPKPKDTLMISRTPEVTCVVVDVSHEDPEVKFNWYVDGVEVHNAKTKPREEQYNSTYRVVSVLTVLHQDWLNGKEYKCKVSNKALPAPIEKTISKAKGQPREPQVYTLPPSREEMTKNQVSLTCLVKGFYPSDIAVEWESNGQPENNYKTTPPVLDSDGSFFLYSKLTVDKSRWQQGNVFSCSVMHEALHNHYTQKSLSLSPGK

SEQ ID NO: 178 - protein, 450 aa, synthetic construct
  REGION 1..450: note = PR003262 HC
QVQLVESGGGVVQPGRSLRLSCAASGFTFSRYGIHWVRQAPGKGLEWVAVIWYNGRNKYYVDSVKGRFTISRDNSKNTLYLQMNSLRAEDTAVYYCARDGGYSYGPFDYWGQGTLVTVSSASTKGPSVFPLAPSSKSTSGGTAALGCLVKDYFPEPVTVSWNSGALTSGVHTFPAVLQSSGLYSLSSVVTVPSSSLGTQTYICNVNHKPSNTKVDKKVEPKSCDKTHTCPPCPAPELLGGPSVFLFPPKPKDTLMISRTPEVTCVVVDVSHEDPEVKFNWYVDGVEVHNAKTKPREEQYNSTYRVVSVLTVLHQDWLNGKEYKCKVSNKALPAPIEKTISKAKGQPREPQVYTLPPSREEMTKNQVSLTCLVKGFYPSDIAVEWESNGQPENNYKTTPPVLDSDGSFFLYSKLTVDKSRWQQGNVFSCSVMHEALHNHYTQKSLSLSPGK

SEQ ID NO: 179 - protein, 453 aa, synthetic construct
  REGION 1..453: note = PR003263 HC
QVQLVESGGGVVQPGRSLRLSCAASGFTFSYYGLNWVRQAPGKGLEWVAVIWFDGTNKYYADSVKGRFTISRDDSKNTLYLQMNSLRAEDTAVYYCARGYGSGSYYNYVMDAWGQGASVTVSSASTKGPSVFPLAPSSKSTSGGTAALGCLVKDYFPEPVTVSWNSGALTSGVHTFPAVLQSSGLYSLSSVVTVPSSSLGTQTYICNVNHKPSNTKVDKKVEPKSCDKTHTCPPCPAPELLGGPSVFLFPPKPKDTLMISRTPEVTCVVVDVSHEDPEVKFNWYVDGVEVHNAKTKPREEQYNSTYRVVSVLTVLHQDWLNGKEYKCKVSNKALPAPIEKTISKAKGQPREPQVYTLPPSREEMTKNQVSLTCLVKGFYPSDIAVEWESNGQPENNYKTTPPVLDSDGSFFLYSKLTVDKSRWQQGNVFSCSVMHEALHNHYTQKSLSLSPGK

SEQ ID NO: 180 - protein, 451 aa, synthetic construct
  REGION 1..451: note = PR003264 HC
QVQLVQSGAEVKKPGSSVKVSCKTSGGTFSSYAISWVRQAPGQGLEWMGGIIPLIGTANYAQNFQGRVTITADESTRTAYMELSSLRSDDTAVYYCARDTMVRGVRALDYWGQGTLVTVSSASTKGPSVFPLAPSSKSTSGGTAALGCLVKDYFPEPVTVSWNSGALTSGVHTFPAVLQSSGLYSLSSVVTVPSSSLGTQTYICNVNHKPSNTKVDKKVEPKSCDKTHTCPPCPAPELLGGPSVFLFPPKPKDTLMISRTPEVTCVVVDVSHEDPEVKFNWYVDGVEVHNAKTKPREEQYNSTYRVVSVLTVLHQDWLNGKEYKCKVSNKALPAPIEKTISKAKGQPREPQVYTLPPSREEMTKNQVSLTCLVKGFYPSDIAVEWESNGQPENNYKTTPPVLDSDGSFFLYSKLTVDKSRWQQGNVFSCSVMHEALHNHYTQKSLSLSPGK

SEQ ID NO: 181 - protein, 451 aa, synthetic construct
  REGION 1..451: note = PR003265 HC
QVQLVESGGGVVQPGRSLRLSCAASGFTFSTYGLHWVRQAPGKGLEWVAVIWYDESNEYYADSVKGRFTISRDNSKNTLYLQMNSLRAEDTALYYCARLAHDYGGTYFDYWGQGTLVTVSSASTKGPSVFPLAPSSKSTSGGTAALGCLVKDYFPEPVTVSWNSGALTSGVHTFPAVLQSSGLYSLSSVVTVPSSSLGTQTYICNVNHKPSNTKVDKKVEPKSCDKTHTCPPCPAPELLGGPSVFLFPPKPKDTLMISRTPEVTCVVVDVSHEDPEVKFNWYVDGVEVHNAKTKPREEQYNSTYRVVSVLTVLHQDWLNGKEYKCKVSNKALPAPIEKTISKAKGQPREPQVYTLPPSREEMTKNQVSLTCLVKGFYPSDIAVEWESNGQPENNYKTTPPVLDSDGSFFLYSKLTVDKSRWQQGNVFSCSVMHEALHNHYTQKSLSLSPGK

SEQ ID NO: 182 - protein, 451 aa, synthetic construct
  REGION 1..451: note = PR003266 HC
QVQLVESGGGVVQPGRSLRLSCAASGFTFSDYGMHWVRQAPGKGLEWVAIIWYDGSNKYYADSVKGRFTISRDNSKNTLYLQMNSLRAEDTAVYYCARDRSSGALGYFQHWGQGTLVTVSSASTKGPSVFPLAPSSKSTSGGTAALGCLVKDYFPEPVTVSWNSGALTSGVHTFPAVLQSSGLYSLSSVVTVPSSSLGTQTYICNVNHKPSNTKVDKKVEPKSCDKTHTCPPCPAPELLGGPSVFLFPPKPKDTLMISRTPEVTCVVVDVSHEDPEVKFNWYVDGVEVHNAKTKPREEQYNSTYRVVSVLTVLHQDWLNGKEYKCKVSNKALPAPIEKTISKAKGQPREPQVYTLPPSREEMTKNQVSLTCLVKGFYPSDIAVEWESNGQPENNYKTTPPVLDSDGSFFLYSKLTVDKSRWQQGNVFSCSVMHEALHNHYTQKSLSLSPGK

SEQ ID NO: 183 - protein, 447 aa, synthetic construct
  REGION 1..447: note = PR004260 HC
QVQLQQSGAELVKPGASVKLSCKASGYTFTSHDINWVRQRPEQGLEWIGWIFPGDGSTKFNEKFKGKATLTTDKSSSTAYIQLSRLTSEDSAVYFCARNSFYSMDYWGQGTSVTVSSASTKGPSVFPLAPSSKSTSGGTAALGCLVKDYFPEPVTVSWNSGALTSGVHTFPAVLQSSGLYSLSSVVTVPSSSLGTQTYICNVNHKPSNTKVDKKVEPKSCDKTHTCPPCPAPEAAGGPSVFLFPPKPKDTLMISRTPEVTCVVVDVSHEDPEVKFNWYVDGVEVHNAKTKPREEQYNSTYRVVSVLTVLHQDWLNGKEYKCKVSNKALPAPIEKTISKAKGQPREPQVYTLPPSREEMTKNQVSLTCLVKGFYPSDIAVEWESNGQPENNYKTTPPVLDSDGSFFLYSKLTVDKSRWQQGNVFSCSVMHEALHNHYTQKSLSLSPGK

SEQ ID NO: 184 - protein, 451 aa, synthetic construct
  REGION 1..451: note = PR004261 HC, PR004485 HC, PR004486 HC
QVQLVESGGGVVQPGRSLRLSCAASGFTFSDYGIHWVRQAPGKGLEWVAVIWYDGSDKYYADSVRGRFTISRDNSKNTLSLQMNSLRVEDTAVYYCARDRSSGAMGYFVYWGQGTLVTVSSASTKGPSVFPLAPSSKSTSGGTAALGCLVKDYFPEPVTVSWNSGALTSGVHTFPAVLQSSGLYSLSSVVTVPSSSLGTQTYICNVNHKPSNTKVDKKVEPKSCDKTHTCPPCPAPEAAGGPSVFLFPPKPKDTLMISRTPEVTCVVVDVSHEDPEVKFNWYVDGVEVHNAKTKPREEQYNSTYRVVSVLTVLHQDWLNGKEYKCKVSNKALPAPIEKTISKAKGQPREPQVYTLPPSREEMTKNQVSLTCLVKGFYPSDIAVEWESNGQPENNYKTTPPVLDSDGSFFLYSKLTVDKSRWQQGNVFSCSVMHEALHNHYTQKSLSLSPGK

SEQ ID NO: 185 - protein, 450 aa, synthetic construct
  REGION 1..450: note = PR004262 HC, PR004493 HC, PR004494 HC
QVQLVESGGGVVQPGRSLRLSCAASGFTFSNYGMHWVRQVPGKGLEWVAVIWYDGSEKDYADSVKGRFTISRDNSKNTLYLQMNSLRVEDTAVYYCAKDLISGIYYVDHWGQGTLVTVSSASTKGPSVFPLAPSSKSTSGGTAALGCLVKDYFPEPVTVSWNSGALTSGVHTFPAVLQSSGLYSLSSVVTVPSSSLGTQTYICNVNHKPSNTKVDKKVEPKSCDKTHTCPPCPAPEAAGGPSVFLFPPKPKDTLMISRTPEVTCVVVDVSHEDPEVKFNWYVDGVEVHNAKTKPREEQYNSTYRVVSVLTVLHQDWLNGKEYKCKVSNKALPAPIEKTISKAKGQPREPQVYTLPPSREEMTKNQVSLTCLVKGFYPSDIAVEWESNGQPENNYKTTPPVLDSDGSFFLYSKLTVDKSRWQQGNVFSCSVMHEALHNHYTQKSLSLSPGK

SEQ ID NO: 186 - protein, 451 aa, synthetic construct
  REGION 1..451: note = PR004263 HC
QVQLVQSGAEVKKPGSSVKVSCKTSGGTFSSYAISWVRQAPGQGLEWMGGIIPLIGTANYAQNFQGRVTITADESTRTAYMELSSLRSDDTAVYYCARDTMVRGVRALDYWGQGTLVTVSSASTKGPSVFPLAPSSKSTSGGTAALGCLVKDYFPEPVTVSWNSGALTSGVHTFPAVLQSSGLYSLSSVVTVPSSSLGTQTYICNVNHKPSNTKVDKKVEPKSCDKTHTCPPCPAPEAAGGPSVFLFPPKPKDTLMISRTPEVTCVVVDVSHEDPEVKFNWYVDGVEVHNAKTKPREEQYNSTYRVVSVLTVLHQDWLNGKEYKCKVSNKALPAPIEKTISKAKGQPREPQVYTLPPSREEMTKNQVSLTCLVKGFYPSDIAVEWESNGQPENNYKTTPPVLDSDGSFFLYSKLTVDKSRWQQGNVFSCSVMHEALHNHYTQKSLSLSPGK

SEQ ID NO: 187 - protein, 451 aa, synthetic construct
  REGION 1..451: note = PR004479 HC, PR004480 HC, PR004481 HC
QVQLVESGGGVVQPGRSLRLSCAASGFTFSDYGIHWVRQAPGKGLEWVAVIWYEGSDKYYADSVRGRFTISRDNSKNTLSLQMNSLRVEDTAVYYCARDRSSGAMGYFVYWGQGTLVTVSSASTKGPSVFPLAPSSKSTSGGTAALGCLVKDYFPEPVTVSWNSGALTSGVHTFPAVLQSSGLYSLSSVVTVPSSSLGTQTYICNVNHKPSNTKVDKKVEPKSCDKTHTCPPCPAPEAAGGPSVFLFPPKPKDTLMISRTPEVTCVVVDVSHEDPEVKFNWYVDGVEVHNAKTKPREEQYNSTYRVVSVLTVLHQDWLNGKEYKCKVSNKALPAPIEKTISKAKGQPREPQVYTLPPSREEMTKNQVSLTCLVKGFYPSDIAVEWESNGQPENNYKTTPPVLDSDGSFFLYSKLTVDKSRWQQGNVFSCSVMHEALHNHYTQKSLSLSPGK

SEQ ID NO: 188 - protein, 451 aa, synthetic construct
  REGION 1..451: note = PR004482 HC, PR004483 HC, PR004484 HC
QVQLVESGGGVVQPGRSLRLSCAASGFTFSDYGIHWVRQAPGKGLEWVAVIWYDASDKYYADSVRGRFTISRDNSKNTLSLQMNSLRVEDTAVYYCARDRSSGAMGYFVYWGQGTLVTVSSASTKGPSVFPLAPSSKSTSGGTAALGCLVKDYFPEPVTVSWNSGALTSGVHTFPAVLQSSGLYSLSSVVTVPSSSLGTQTYICNVNHKPSNTKVDKKVEPKSCDKTHTCPPCPAPEAAGGPSVFLFPPKPKDTLMISRTPEVTCVVVDVSHEDPEVKFNWYVDGVEVHNAKTKPREEQYNSTYRVVSVLTVLHQDWLNGKEYKCKVSNKALPAPIEKTISKAKGQPREPQVYTLPPSREEMTKNQVSLTCLVKGFYPSDIAVEWESNGQPENNYKTTPPVLDSDGSFFLYSKLTVDKSRWQQGNVFSCSVMHEALHNHYTQKSLSLSPGK

SEQ ID NO: 189 - protein, 450 aa, synthetic construct
  REGION 1..450: note = PR004487 HC, PR004488 HC, PR004489 HC
QVQLVESGGGVVQPGRSLRLSCAASGFTFSNYGMHWVRQVPGKGLEWVAVIWYEGSEKDYADSVKGRFTISRDNSKNTLYLQMNSLRVEDTAVYYCAKDLISGIYYVDHWGQGTLVTVSSASTKGPSVFPLAPSSKSTSGGTAALGCLVKDYFPEPVTVSWNSGALTSGVHTFPAVLQSSGLYSLSSVVTVPSSSLGTQTYICNVNHKPSNTKVDKKVEPKSCDKTHTCPPCPAPEAAGGPSVFLFPPKPKDTLMISRTPEVTCVVVDVSHEDPEVKFNWYVDGVEVHNAKTKPREEQYNSTYRVVSVLTVLHQDWLNGKEYKCKVSNKALPAPIEKTISKAKGQPREPQVYTLPPSREEMTKNQVSLTCLVKGFYPSDIAVEWESNGQPENNYKTTPPVLDSDGSFFLYSKLTVDKSRWQQGNVFSCSVMHEALHNHYTQKSLSLSPGK

SEQ ID NO: 190 - protein, 450 aa, synthetic construct
  REGION 1..450: note = PR004490 HC, PR004491 HC, PR004492 HC
QVQLVESGGGVVQPGRSLRLSCAASGFTFSNYGMHWVRQVPGKGLEWVAVIWYDASEKDYADSVKGRFTISRDNSKNTLYLQMNSLRVEDTAVYYCAKDLISGIYYVDHWGQGTLVTVSSASTKGPSVFPLAPSSKSTSGGTAALGCLVKDYFPEPVTVSWNSGALTSGVHTFPAVLQSSGLYSLSSVVTVPSSSLGTQTYICNVNHKPSNTKVDKKVEPKSCDKTHTCPPCPAPEAAGGPSVFLFPPKPKDTLMISRTPEVTCVVVDVSHEDPEVKFNWYVDGVEVHNAKTKPREEQYNSTYRVVSVLTVLHQDWLNGKEYKCKVSNKALPAPIEKTISKAKGQPREPQVYTLPPSREEMTKNQVSLTCLVKGFYPSDIAVEWESNGQPENNYKTTPPVLDSDGSFFLYSKLTVDKSRWQQGNVFSCSVMHEALHNHYTQKSLSLSPGK

SEQ ID NO: 191 - protein, 219 aa, synthetic construct
  REGION 1..219: note = PR003181 LC, PR004260 LC
DIVMSQSPSSLAVSAGEKVTMSCKSSQSLLNSRTRKNQLAWYQQKPGQSPKLLIYWASTRESGVPDRFTGSGSGTDFTLTISSVQAEDLAVYYCKQSYNLRTFGGGTKLEIKRTVAAPSVFIFPPSDEQLKSGTASVVCLLNNFYPREAKVQWKVDNALQSGNSQESVTEQDSKDSTYSLSSTLTLSKADYEKHKVYACEVTHQGLSSPVTKSFNRGEC

SEQ ID NO: 192 - protein, 213 aa, synthetic construct
  REGION 1..213: note = PR003248 LC
DIQMTQSPSTLSASVGDRVTITCRASQSINNWLAWYQQKPGKAPKLLIYKASSLESGVPSRFSGSGSGTEFTLTISSLQPDDFATYYCQQYNSYSTFGQGTKLEIKRTVAAPSVFIFPPSDEQLKSGTASVVCLLNNFYPREAKVQWKVDNALQSGNSQESVTEQDSKDSTYSLSSTLTLSKADYEKHKVYACEVTHQGLSSPVTKSFNRGEC

SEQ ID NO: 193 - protein, 214 aa, synthetic construct
  REGION 1..214: note = PR003249 LC, PR003250 LC, PR004261 LC, PR004479 LC, PR004482 LC
DIQMTQSPSTLSASVGDRVTITCRASQSISSWLAWYQQKPGKAPKLLIYKASSLESGVPSRFSGSGSGTEFTLTISSLQPDDLATYYCQQYNSYSYTFGQGTKLEIKRTVAAPSVFIFPPSDEQLKSGTASVVCLLNNFYPREAKVQWKVDNALQSGNSQESVTEQDSKDSTYSLSSTLTLSKADYEKHKVYACEVTHQGLSSPVTKSFNRGEC

SEQ ID NO: 194 - protein, 214 aa, synthetic construct
  REGION 1..214: note = PR003251 LC
EIVMTQSPATLSVSPGEGATLSCRASQSVSSNLAWYQQKPGQAPRLLIYGASTRATGIPARFSGSGSGTEFTLTISSLQSEDFAVYYCQQYNIWPYTFGQGTKLEIKRTVAAPSVFIFPPSDEQLKSGTASVVCLLNNFYPREAKVQWKVDNALQSGNSQESVTEQDSKDSTYSLSSTLTLSKADYEKHKVYACEVTHQGLSSPVTKSFNRGEC

SEQ ID NO: 195 - protein, 213 aa, synthetic construct
  REGION 1..213: note = PR003252 LC
DIQMTQSPSTLSASVGDRVTITCRASQSISSWLAWYQQKPGKAPKLLIYKASSLKSGVPSRFSGSGSGTEFTLTISSLQPDDFATYYCLQYNSYYTFGQGTKLEIKRTVAAPSVFIFPPSDEQLKSGTASVVCLLNNFYPREAKVQWKVDNALQSGNSQESVTEQDSKDSTYSLSSTLTLSKADYEKHKVYACEVTHQGLSSPVTKSFNRGEC

SEQ ID NO: 196 - protein, 214 aa, synthetic construct
  REGION 1..214: note = PR003254 LC
EIVMTQSPATLSVSPGERATLSCRASQSVSSYLAWYQQKPGQAPRLLIYGASTRATGIPARFSGSGSGTEFTLTISSLQSEDFAVYYCQQYNNWPLTFGGGTKVEIKRTVAAPSVFIFPPSDEQLKSGTASVVCLLNNFYPREAKVQWKVDNALQSGNSQESVTEQDSKDSTYSLSSTLTLSKADYEKHKVYACEVTHQGLSSPVTKSFNRGEC

SEQ ID NO: 197 - protein, 214 aa, synthetic construct
  REGION 1..214: note = PR003259 LC, PR004262 LC, PR004487 LC, PR004490 LC
DIQMTQSPSSLSASVGDRVTITCRASQGISNYLAWYQQKPGKVPKLLIYAASTLQSGVPSRFSGSGSGTDFTLTISSLQPEDVATYYCQKYNSAPFTFGPGTKVDIKRTVAAPSVFIFPPSDEQLKSGTASVVCLLNNFYPREAKVQWKVDNALQSGNSQESVTEQDSKDSTYSLSSTLTLSKADYEKHKVYACEVTHQGLSSPVTKSFNRGEC

SEQ ID NO: 198 - protein, 214 aa, synthetic construct
  REGION 1..214: note = PR003260 LC
EIVMTQSPATLSVSPGERATLSCRASQSVSSNLAWYQQKPGQAPRLLIYYASTRAPGIPARFSGSESGTEFTLTISSLQSEDFAVYYCQQYNIWPYTFGQGTKLEIKRTVAAPSVFIFPPSDEQLKSGTASVVCLLNNFYPREAKVQWKVDNALQSGNSQESVTEQDSKDSTYSLSSTLTLSKADYEKHKVYACEVTHQGLSSPVTKSFNRGEC

SEQ ID NO: 199 - protein, 214 aa, synthetic construct
  REGION 1..214: note = PR003261 LC
DIQMTQSPSTLSASVGDRVTITCRASQSISSWLAWYQQKPGKAPKLLIYKASSLESGVPSRFSGSGSGTEFTLTISSLQPDDFASYYCQQYNSYSVTFGGGTKVEIKRTVAAPSVFIFPPSDEQLKSGTASVVCLLNNFYPREAKVQWKVDNALQSGNSQESVTEQDSKDSTYSLSSTLTLSKADYEKHKVYACEVTHQGLSSPVTKSFNRGEC

SEQ ID NO: 200 - protein, 214 aa, synthetic construct
  REGION 1..214: note = PR003262 LC
EIVMTQSPATLSVSPGERATLSCRASQSFSNNLAWYQQKPGQAPRLLIYGASTRATGIPARFSGSGSGTEFTLTISSLQSEDFAVYYCHQYNIWPLTFGGGTKVEIKRTVAAPSVFIFPPSDEQLKSGTASVVCLLNNFYPREAKVQWKVDNALQSGNSQESVTEQDSKDSTYSLSSTLTLSKADYEKHKVYACEVTHQGLSSPVTKSFNRGEC

SEQ ID NO: 201 - protein, 214 aa, synthetic construct
  REGION 1..214: note = PR003263 LC
EIVMTQSPATLSVSPGERATLSCRASQSVSSNLAWYQQKPGQAPRLLIYGASTGATGIPARFSGSGSGTDFTLTISSLQSEDFAVYYCQQYYKWPLTFGGGTKVEIKRTVAAPSVFIFPPSDEQLKSGTASVVCLLNNFYPREAKVQWKVDNALQSGNSQESVTEQDSKDSTYSLSSTLTLSKADYEKHKVYACEVTHQGLSSPVTKSFNRGEC

SEQ ID NO: 202 - protein, 214 aa, synthetic construct
  REGION 1..214: note = PR003264 LC, PR004263 LC
DIQLTQSPSFLSASVGDRVTITCRASQGISSYFAWYQQKPGKAPKLLIYAASTLQSGVPSRFSGSGSGTEFTLTISSLQPEDFATYYCQHLNRYPWTFGQGTKVEIKRTVAAPSVFIFPPSDEQLKSGTASVVCLLNNFYPREAKVQWKVDNALQSGNSQESVTEQDSKDSTYSLSSTLTLSKADYEKHKVYACEVTHQGLSSPVTKSFNRGEC

SEQ ID NO: 203 - protein, 215 aa, synthetic construct
  REGION 1..215: note = PR003265 LC
EIVMTQSPAILSVSPGERATLSCRASQSISYNLAWYQQKPGQAPRLLIYGASIRATGIPARFSGSGSGTDFTLTISSLQSEDFAVYYCQQYNNWPPWTFGQGTKVEIKRTVAAPSVFIFPPSDEQLKSGTASVVCLLNNFYPREAKVQWKVDNALQSGNSQESVTEQDSKDSTYSLSSTLTLSKADYEKHKVYACEVTHQGLSSPVTKSFNRGEC

SEQ ID NO: 204 - protein, 213 aa, synthetic construct
  REGION 1..213: note = PR003266 LC
DIQMTQSPSTLSASVGDRVTITCRASQSISSWLAWYQQKPGKAPKLLIYKASSLESGVPSRFSGSGSGTEFTLTISSLQPDDFATYYCQQYNSYSTFGQGTKLEIKRTVAAPSVFIFPPSDEQLKSGTASVVCLLNNFYPREAKVQWKVDNALQSGNSQESVTEQDSKDSTYSLSSTLTLSKADYEKHKVYACEVTHQGLSSPVTKSFNRGEC

SEQ ID NO: 205 - protein, 214 aa, synthetic construct
  REGION 1..214: note = PR004480 LC, PR004483 LC, PR004485 LC
DIQMTQSPSTLSASVGDRVTITCRASQSISSWLAWYQQKPGKAPKLLIYKASSLESGVPSRFSGSGSGTEFTLTISSLQPDDLATYYCQQYQSYSYTFGQGTKLEIKRTVAAPSVFIFPPSDEQLKSGTASVVCLLNNFYPREAKVQWKVDNALQSGNSQESVTEQDSKDSTYSLSSTLTLSKADYEKHKVYACEVTHQGLSSPVTKSFNRGEC

SEQ ID NO: 206 - protein, 214 aa, synthetic construct
  REGION 1..214: note = PR004481 LC, PR004484 LC, PR004486 LC
DIQMTQSPSTLSASVGDRVTITCRASQSISSWLAWYQQKPGKAPKLLIYKASSLESGVPSRFSGSGSGTEFTLTISSLQPDDLATYYCQQYNAYSYTFGQGTKLEIKRTVAAPSVFIFPPSDEQLKSGTASVVCLLNNFYPREAKVQWKVDNALQSGNSQESVTEQDSKDSTYSLSSTLTLSKADYEKHKVYACEVTHQGLSSPVTKSFNRGEC

SEQ ID NO: 207 - protein, 214 aa, synthetic construct
  REGION 1..214: note = PR004488 LC, PR004491 LC, PR004493 LC
DIQMTQSPSSLSASVGDRVTITCRASQGISNYLAWYQQKPGKVPKLLIYAASTLQSGVPSRFSGSGSGTDFTLTISSLQPEDVATYYCQKYQSAPFTFGPGTKVDIKRTVAAPSVFIFPPSDEQLKSGTASVVCLLNNFYPREAKVQWKVDNALQSGNSQESVTEQDSKDSTYSLSSTLTLSKADYEKHKVYACEVTHQGLSSPVTKSFNRGEC

SEQ ID NO: 208 - protein, 214 aa, synthetic construct
  REGION 1..214: note = PR004489 LC, PR004492 LC, PR004494 LC
DIQMTQSPSSLSASVGDRVTITCRASQGISNYLAWYQQKPGKVPKLLIYAASTLQSGVPSRFSGSGSGTDFTLTISSLQPEDVATYYCQKYNAAPFTFGPGTKVDIKRTVAAPSVFIFPPSDEQLKSGTASVVCLLNNFYPREAKVQWKVDNALQSGNSQESVTEQDSKDSTYSLSSTLTLSKADYEKHKVYACEVTHQGLSSPVTKSFNRGEC